European Patent Application EP 4 606 907 A1, published August 27, 2025. Title: BIOLOGICAL SUBSTANCE TREATMENT METHOD, REACTION DETECTION METHOD, BIOLOGICAL SUBSTANCE TREATMENT APPARATUS, AND REACTION DETECTION APPARATUS. Applicant: JAPAN SCIENCE AND TECHNOLOGY AGENCY. Application EP 23879775.7, filed October 17, 2023. The sequence listing filed with the application follows.

SEQUENCE LISTING (2 sequences)

SEQ ID NO: 1 - RNA, 3001 nt, synthetic construct
  source 1..3001: mol_type = other RNA; note = RNA containing a sequence encoding the S gene fragment of SERS-CoV-2
gggtaacatcactaggtttcaaactttacttgctttacatagaagttatttgactcctggtgattcttcttcaggttggacagctggtgctgcagcttattatgtgggttatcttcaacctagggagaacagcaagaagcacgagaagtacaagatccgcgagtactatcacaagatcatcggccggaagaacgacaaagagaacttcgccaagattatctacgaagagatccagaacgtgaacaacatcaaagagctgattgagaagatccccgacatgtctgagctgaagaaaagccaggtgttctacaagtactacctggacaaagaggaactgaacgacaagaatattaagtacgccttctgccacttcgtggaaatcgagatgtcccagctgctgaaaaactacgtgtacaagcggctgagcaacatcagcaacgataagatcaagcggatcttcgagtaccagaatctgaaaaagctgatcgaaaacaaactgctgaacaagctggacacctacgtgcggaactgcggcaagtacaactactatctgcaagtgggcgagatcgccacctccgactttatcgcccggaaccggcagaacgaggccttcctgagaaacatcatcggcgtgtccagcgtggcctacttcagcctgaggaacatcctggaaaccgagaacgagaacgatatcaccggccggatgcggggcaagaccgtgaagaacaacaagggcgaagagaaatacgtgtccggcgaggtggacaagatctacaatgagaacaagcagaacgaagtgaaagaaaatctgaagatgttctacagctacgacttcaacatggacaacaagaacgagatcgaggacttcttcgccaacatcgacgaggccatcagcagcatcagacacggcatcgtgcacttcaacctggaactggaaggcaaggacatcttcgccttcaagaatatcgcccccagcgagatctccaagaagatgtttcagaacgaaatcaacgaaaagaagctgaagctgaaaatcttcaagcagctgaacagcgccaacgtgttcaactactacgagaaggatgtgatcatcaagtacctgaagaataccaagttcaacttcgtgaacaaaaacatccccttcgtgcccagcttcaccaagctgtacaacaagattgaggacctgcggaataccctgaagtttttttggagcgtgcccaaggacaaagaagagaaggacgcccagatctacctgctgaagaatatctactacggcgagttcctgaacaagttcgtgaaaaactccaaggtgttctttaagatcaccaatgaagtgatcaagattaacaagcagcggaaccagaaaaccggccactacaagtatcagaagttcgagaacatcgagaaaaccgtgcccgtggaatacctggccatcatccagagcagagagatgatcaacaaccaggacaaagaggaaaagaatacctacatcgactttattcagcagattttcctgaagggcttcatcgactacctgaacaagaacaatctgaagtatatcgagagcaacaacaacaatgacaacaacgacatcttctccaagatcaagatcaaaaaggataacaaagagaagtacgacaagatcctgaagaactatgagaagcacaatcggaacaaagaaatccctcacgagatcaatgagttcgtgcgcgagatcaagctggggaagattctgaagtacaccgagaatctgaacatgttttacctgatcctgaagctgctgaaccacaaagagctgaccaacctgaagggcagcctggaaaagtaccagtccgccaacaaagaagaaaccttcagcgacgagctggaactgatcaacctgctgaacctggacaacaacagagtgaccgaggacttcgagctggaagccaacgagatcggcaagttcctggacttcaacgaaaacaaaatcaaggaccggaaagagctgaaaaagttcgacaccaacaagatctatttcgacggcgagaacatcatcaagcaccgggccttctacaatatcaagaaatacggcatgctgaatctgctggaaaagatcgccgataaggccaagtataagatcagcctgaaagaactgaaagagtacagcaacaagaagaatgagattgaaaagaactacaccatgcagcagaacctgcaccggaagtacgccagacccaagaaggacgaaaagttcaacgacgaggactacaaagagtatgagaaggccatcggcaacatccagaagtacacccacctgaagaacaaggtggaattcaatgagctgaacctgctgcagggcctgctgctgaagatcctgcaccggctcgtgggctacaccagcatctgggagcgggacctgagattccggctgaagggcgagtttcccgagaaccactacatcgaggaaattttcaatttcgacaactccaagaatgtgaagtacaaaagcggccagatcgtggaaaagtatatcaacttctacaaagaactgtacaaggacaatgtggaaaagcggagcatctactccgacaagaaagtgaagaaactgaagcaggaaaaaaaggacctgtacatccggaactacattgcccacttcaactacatcccccacgccgagattagcctgctggaagtgctggaaaacctgcggaagctgctgtcctacgaccggaagctgaagaacgccatcatgaagtccatcgtggacattctgaaagaatacggcttcgtggccaccttcaagatcggcgctgacaagaagatcgaaatccagaccctggaatcagagaagatcgtgcacctgaagaatctgaagaaaaagaaactgatgaccgaccggaacagcgaggaactgtgcgaactcgtgaaagtcatgttcgagtacaaggccctggaataagcggccgcactcgaggcccgaaaggaagctgagttggctgctgccaccgctgagcaataa

SEQ ID NO: 2 - RNA, 64 nt, synthetic construct
  source 1..64: mol_type = other RNA
gatttagactaccccaaaaacgaaggggactaaaacgcagcaccagctgtccaacctgaagaag